European Patent Application EP 4 582 446 A2, published July 9, 2025. Title: AN ANTIBODY FOR USE IN METHODS OF TREATING AL AMYLOIDOSIS. Applicant: PROTHENA BIOSCIENCES LIMITED. Application EP. The sequence listing filed with the application follows.

SEQUENCE LISTING (23 sequences)

SEQ ID NO: 1 - protein, 112 aa, synthetic construct
  REGION 1..112: note = Synthetic peptide
DVVMTQSPLSLPVTPGEPASISCRSSQSLVHSTGNTYLHWYLQKPGQSPQLLIYKVSNRFSGVPDRFSGSGSGTDFTLKISRVEAEDVGVYYCSQSTHVPFTFGGGTKVEIK

SEQ ID NO: 2 - protein, 119 aa, synthetic construct
  REGION 1..119: note = Synthetic peptide
EVQLVESGGGLVQPGGSLRLSCAASGFTFNTYAMYWIRQAPGKGLEWVARIRSKSNNYAIYYADSVKDRFTISRDDSKNSLYLQMNSLKTEDTAVYYCARPYSDSFAYWGQGTLVTVSS

SEQ ID NO: 3 - protein, 16 aa, synthetic construct
  REGION 1..16: note = Synthetic peptide
RSSQSLVHSTGNTYLH

SEQ ID NO: 4 - protein, 7 aa, synthetic construct
  REGION 1..7: note = Synthetic peptide
KVSNRFS

SEQ ID NO: 5 - protein, 9 aa, synthetic construct
  REGION 1..9: note = Synthetic peptide
SQSTHVPFT

SEQ ID NO: 6 - protein, 10 aa, synthetic construct
  REGION 1..10: note = Synthetic peptide
GFTFNTYAMY

SEQ ID NO: 7 - protein, 19 aa, synthetic construct
  REGION 1..19: note = Synthetic peptide
RIRSKSNNYAIYYADSVKD

SEQ ID NO: 8 - protein, 8 aa, synthetic construct
  REGION 1..8: note = Synthetic peptide
PYSDSFAY

SEQ ID NO: 9 - protein, 16 aa, synthetic construct
  REGION 1..16: note = Synthetic peptide
RSSLSLVHSTGNTYLH

SEQ ID NO: 10 - protein, 219 aa, synthetic construct
  REGION 1..219: note = Synthetic peptide
DVVMTQSPLSLPVTPGEPASISCRSSQSLVHSTGNTYLHWYLQKPGQSPQLLIYKVSNRFSGVPDRFSGSGSGTDFTLKISRVEAEDVGVYYCSQSTHVPFTFGGGTKVEIKRTVAAPSVFIFPPSDEQLKSGTASVVCLLNNFYPREAKVQWKVDNALQSGNSQESVTEQDSKDSTYSLSSTLTLSKADYEKHKVYACEVTHQGLSSPVTKSFNRGEC

SEQ ID NO: 11 - protein, 449 aa, synthetic construct
  REGION 1..449: note = Synthetic peptide
EVQLVESGGGLVQPGGSLRLSCAASGFTFNTYAMYWIRQAPGKGLEWVARIRSKSNNYAIYYADSVKDRFTISRDDSKNSLYLQMNSLKTEDTAVYYCARPYSDSFAYWGQGTLVTVSSASTKGPSVFPLAPSSKSTSGGTAALGCLVKDYFPEPVTVSWNSGALTSGVHTFPAVLQSSGLYSLSSVVTVPSSSLGTQTYICNVNHKPSNTKVDKRVEPKSCDKTHTCPPCPAPELLGGPSVFLFPPKPKDTLMISRTPEVTCVVVDVSHEDPEVKFNWYVDGVEVHNAKTKPREEQYNSTYRVVSVLTVLHQDWLNGKEYKCKVSNKALPAPIEKTISKAKGQPREPQVYTLPPSRDELTKNQVSLTCLVKGFYPSDIAVEWESNGQPENNYKTTPPVLDSDGSFFLYSKLTVDKSRWQQGNVFSCSVMHEALHNHYTQKSLSLSPGK

SEQ ID NO: 12 - protein, 449 aa, synthetic construct
  REGION 1..449: note = Synthetic peptide
EVQLVESGGGLVQPGGSLRLSCAASGFTFNTYAMYWIRQAPGKGLEWVARIRSKSNNYAIYYADSVKDRFTISRDDSKNSLYLQMNSLKTEDTAVYYCARPYSDSFAYWGQGTLVTVSSASTKGPSVFPLAPSSKSTSGGTAALGCLVKDYFPEPVTVSWNSGALTSGVHTFPAVLQSSGLYSLSSVVTVPSSSLGTQTYICNVNHKPSNTKVDKRVEPKSCDKTHTCPPCPAPELLGGPSVFLFPPKPKDTLMISRTPEVTCVVVDVSHEDPEVKFNWYVDGVEVHNAKTKPREEQYNSTYRVVSVLTVLHQDWLNGKEYKCKVSNKALPAPIEKTISKAKGQPREPQVYTLPPSREEMTKNQVSLTCLVKGFYPSDIAVEWESNGQPENNYKTTPPVLDSDGSFFLYSKLTVDKSRWQQGNVFSCSVMHEALHNHYTQKSLSLSPGK

SEQ ID NO: 13 - protein, 445 aa, synthetic construct
  REGION 1..445: note = Synthetic peptide
EVQLVESGGGLVQPGGSLRLSCAASGFTFNTYAMYWIRQAPGKGLEWVARIRSKSNNYAIYYADSVKDRFTISRDDSKNSLYLQMNSLKTEDTAVYYCARPYSDSFAYWGQGTLVTVSSASTKGPSVFPLAPCSRSTSESTAALGCLVKDYFPEPVTVSWNSGALTSGVHTFPAVLQSSGLYSLSSVVTVPSSNFGTQTYTCNVDHKPSNTKVDKTVERKCCVECPPCPAPPVAGPSVFLFPPKPKDTLMISRTPEVTCVVVDVSHEDPEVQFNWYVDGVEVHNAKTKPREEQFNSTFRVVSVLTVVHQDWLNGKEYKCKVSNKGLPAPIEKTISKTKGQPREPQVYTLPPSREEMTKNQVSLTCLVKGFYPSDIAVEWESNGQPENNYKTTPPMLDSDGSFFLYSKLTVDKSRWQQGNVFSCSVMHEALHNHYTQKSLSLSPGK

SEQ ID NO: 14 - protein, 112 aa, synthetic construct
  REGION 1..112: note = Synthetic peptide
DVVMTQTPLSLPVSLGDQASISCRSSQSLVHRNGNTYLHWYLQKPGQSPKLLIYKVSNRFSGVPDRFSGSGSGTDFTLKISRVEAEDLGLYFCFQTTYVPNTFGGGTKLEIK

SEQ ID NO: 15 - protein, 111 aa, synthetic construct
  REGION 1..111: note = Synthetic peptide
QVQLKESGPGLVAPSQSLSITCTVSGFSLSSYGVSWVRQPPGKGLEWLGVIWGDGSTNYKPNLMSRLSISKDISKSQVLFKLNSLQTDDTATYYCVTLDYWGQGTSVTVSS

SEQ ID NO: 16 - protein, 16 aa, synthetic construct
  REGION 1..16: note = Synthetic peptide
RSSQSLVHRNGNYTLH

SEQ ID NO: 17 - protein, 7 aa, synthetic construct
  REGION 1..7: note = Synthetic peptide
LVSNRFS

SEQ ID NO: 18 - protein, 9 aa, synthetic construct
  REGION 1..9: note = Synthetic peptide
FNTTYVPNT

SEQ ID NO: 19 - protein, 6 aa, synthetic construct
  REGION 1..6: note = Synthetic peptide
SYGVSW

SEQ ID NO: 20 - protein, 21 aa, synthetic construct
  REGION 1..21: note = Synthetic peptide
VIWGDGSTNYHPNLMSRLSIS

SEQ ID NO: 21 - skipped

SEQ ID NO: 22 - DNA, 336 bp, synthetic construct
  misc_feature 1..336: note = 11-1F4 monoclonal antibody variable light
  source 1..336: mol_type = other DNA
gatgttgtgatgacccaaactccactctccctgcctgtcagtcttggagatcaagcctccatctcttgcagatctagtcagagccttgtacatagaaatggaaacacctatttacattggtacctgcagaagccaggccagtctccaaagctcctgatctacaaagtttccaaccgattttctggggtcccagacaggttcagtggcagtggatcagggacagatttcacactcaagatcagcagagtggaggctgaggatttgggactttatttctgttttcaaactacatatgttccgaacacgttcggaggggggaccaagctggaaataaaa

SEQ ID NO: 23 - DNA, 333 bp, synthetic construct
  misc_feature 1..333: note = 11-1F4 monoclonal antibody variable heavy
  source 1..333: mol_type = other DNA
caggtgcagctgaaggagtcaggacctggcctggtggcgccctcacagagcctgtccatcacatgcactgtctcagggttctcattaagcagctatggtgtaagctgggttcgccagcctccaggaaagggtctggagtggctgggagtaatatggggtgacgggagcacaaattatcatccaaatctcatgtccagactgagtatcagcaaggatatttccaagagccaagttctcttcaaactgaatagtctgcaaactgatgacacagccacgtactactgtgtcaccttcgactactggggtcaaggaacctcagtcaccgtctcctca